European Patent Specification EP 3 543 359 B1, published February 14, 2024. Title: Molecular Marker and Kit for Early Diagnosis and Prediction of Sepsis Acute Kidney Injury and Application thereof. Applicant: The Second Xiangya Hospital of Central South University. The sequence listing filed with the application follows.

SEQUENCE LISTING (5 sequences)

SEQ ID NO: 1 - RNA, 1611 nt, Sequence of TCONS_00024536
cuuuuuuuucccccugagauggagucucacucuaucgcccaggcuggagugcggugcaguggcauggucuuggcucacugcaaccuccaccuccuggguucaagcaauucuccugccucagccccccaaguagcugggacuauaggcaugccccaccacgcccagauuauuuuuguauuuuuaguagagacaggguuucaccauauuggccaggcuggucucgaacuccugaccucaagaucugcccaccuuggccucccaaagugcugggauuacaggcgugagcuacuaugcccagccuguccaccucuuccuuuagcaaacaaaaucccugggcgaccagagugaccccagaaauuggaggagggcagagaccccgucuuuggaggugauguggaggguguccaggcccgcccuugucucacaggcgcacacccugcuggaggccaagugucggacaugaaggugacgcugccccaugcuguccagacacccagcaaugcucagcacccggaaacaggaccggccucugcucugcguggagcccacccggacaguccaucucagccccuucuacccagggacccccaggccccugcccgcaugcaggaacuguccucugggcagagcagcccccuccccaugagggucucgcaggcccaggacucgcguccagcagcuccuggacauggccuugcugcccggccagggcuaguguccgugaacagagaauagugugugugagcggcucugucaucugucacuuggggcugccugugucccucuccaggaccucagugccgaucgcaggaaaggauguuggcacggcccccggugggacaggccagccacguuaggggaugcugcacgacaaagcccacggcgguggugucacaugaaugucaccugcucuucacacccagccuaggaagggcuguugacuggaggcugacauacccagcgaggccucugacgucccugucacccccuggggugggagaguccccucuuccagccugucuggggccuugccccucccuacagcccagcucgggaaacaaaugcuccuuccagcagcagcagagagcuguagagccggggcuccgggcagcuucugaauccagcucccaggccacagaucacagggacaggacgggagccucccacacagacgccaggcagcaggaccccggcugggaagucacauccaaaggacagaaccaccugcccaaguccccuccacuucugagaaccaccugcccaaguccccuccacgucugagaaccaccugcccaaguccccuccacaucugaacacucauugcuguguccggacgcagaaauucacacucggauuuuguccggcauucccacucccugcccugcuuggagaggcaggaccgcaggucugccggccccaacggcagcgccacagugcccggcacagaggccugcuggucgcgcauacaaagcacccgccggccauuaucauuccggagccggccagagccucccggcugcaucucaucggucauucagcagcccguaaugacuugucaguuccuugcccugccauuuucugucuaauuaauucuuuuauugugcaccggau

SEQ ID NO: 2 - DNA, 20 bp, Primer F for specific amplification of TCONS_00024536
taggaagggctgttgactgg

SEQ ID NO: 3 - DNA, 20 bp, Primer R for specific amplification of TCONS_00024536
ctgggagctggattcagaag

SEQ ID NO: 4 - DNA, 23 bp, Gapdh gene primer F
caaggtcatccatgacaactttg

SEQ ID NO: 5 - DNA, 22 bp, Gapdh gene primer R
gtccaccaccctgttgctgtag